European Patent Specification EP 3 722 310 B1, published August 28, 2024. Title: Stable and soluble antibodies inhibiting VEGF. Applicant: Novartis AG. Application not yet assigned. The sequence listing filed with the application follows.

SEQUENCE LISTING (180 sequences)

SEQ ID NO: 1 - protein, 11 aa, Homo sapiens
KFMDVYQRSYC

SEQ ID NO: 2 - protein, 11 aa, Unknown
  CDR stemming from rabbit antibody
GFPFSSGYWVC

SEQ ID NO: 3 - protein, 11 aa, Unknown
  CDR stemming from rabbit antibody
GFSFSSGYWIC

SEQ ID NO: 4 - protein, 11 aa, Unknown
  CDR stemming from rabbit antibody
GFSLNTNYWMC

SEQ ID NO: 5 - protein, 11 aa, Unknown
  CDR stemming from rabbit antibody
GFSFSRSYYIY

SEQ ID NO: 6 - protein, 11 aa, Unknown
  CDR stemming from rabbit antibody
GFSFTTTDYMC

SEQ ID NO: 7 - protein, 11 aa, Unknown
  CDR stemming from rabbit antibody
GIDFSGAYYMG

SEQ ID NO: 8 - protein, 11 aa, Unknown
  CDR stemming from rabbit antibody
GFSLTDYYYMT

SEQ ID NO: 9 - protein, 10 aa, Unknown
  CDR stemming from rabbit antibody
GFSLSYYYMS

SEQ ID NO: 10 - protein, 10 aa, Unknown
  CDR stemming from rabbit antibody
GFSLSDYYMC

SEQ ID NO: 11 - protein, 10 aa, Unknown
  CDR stemming from rabbit antibody
GFSLSSYYMC

SEQ ID NO: 12 - protein, 10 aa, Unknown
  CDR stemming from rabbit antibody
GFSLNTYYMN

SEQ ID NO: 13 - protein, 10 aa, Unknown
  CDR stemming from rabbit antibody
GFSLSSYYMS

SEQ ID NO: 14 - protein, 11 aa, Unknown
  CDR stemming from rabbit antibody
GFSLSSGYYMC

SEQ ID NO: 15 - protein, 18 aa, Unknown
  CDR stemming from rabbit antibody
CIYAGSSGSTYYASWAKG

SEQ ID NO: 16 - protein, 18 aa, Unknown
  CDR stemming from rabbit antibody
CMYTGSYNRAYYASWAKG

SEQ ID NO: 17 - protein, 18 aa, Unknown
  CDR stemming from rabbit antibody
CIDAGSSGILVYANWAKG

SEQ ID NO: 18 - protein, 17 aa, Unknown
  CDR stemming from rabbit antibody
CILAGDGSTYYANWAKG

SEQ ID NO: 19 - protein, 16 aa, Unknown
  CDR stemming from rabbit antibody
YIDYDGDRYYASWAKG

SEQ ID NO: 20 - protein, 16 aa, Unknown
  CDR stemming from rabbit antibody
FIDPDDDPYYATWAKG

SEQ ID NO: 21 - protein, 16 aa, Unknown
  CDR stemming from rabbit antibody
IIGPGDYTDYASWAKG

SEQ ID NO: 22 - protein, 16 aa, Unknown
  CDR stemming from rabbit antibody
CLDYFGSTDDASWAKG

SEQ ID NO: 23 - protein, 16 aa, artificial sequence
  CDR stemming from rabbit antibody
CLDYVGDTDYASWAKG

SEQ ID NO: 24 - protein, 16 aa, Unknown
  CDR stemming from rabbit antibody
IIAPDDTTYYASWAKS

SEQ ID NO: 25 - protein, 16 aa, Unknown
  CDR stemming from rabbit antibody
ILDYVGDTDYASWAKG

SEQ ID NO: 26 - protein, 18 aa, Unknown
  CDR stemming from rabbit antibody
CIDAGSDGDTYYASWAKG

SEQ ID NO: 27 - protein, 19 aa, Unknown
  CDR stemming from rabbit antibody
GNNYYIYTDGGYAYAGLEL

SEQ ID NO: 28 - protein, 8 aa, Unknown
  CDR stemming from rabbit antibody
GSNWYSDL

SEQ ID NO: 29 - protein, 14 aa, Unknown
  CDR stemming from rabbit antibody
GDASYGVDSFMLPL

SEQ ID NO: 30 - protein, 11 aa, Unknown
  CDR stemming from rabbit antibody
SDPASSWSFAL

SEQ ID NO: 31 - protein, 11 aa, Unknown
  CDR stemming from rabbit antibody
SDYSSGWGTDI

SEQ ID NO: 32 - protein, 11 aa, Unknown
  CDR stemming from rabbit antibody
GDHNSGWGLDI

SEQ ID NO: 33 - protein, 11 aa, Unknown
  CDR stemming from rabbit antibody
GDDNSGWGEDI

SEQ ID NO: 34 - protein, 11 aa, Unknown
  CDR stemming from rabbit antibody
TDDSRGWGLNI

SEQ ID NO: 35 - protein, 11 aa, Unknown
  CDR stemming from rabbit antibody
TDDSRGWGLNI

SEQ ID NO: 36 - protein, 11 aa, Unknown
  CDR stemming from rabbit antibody
SGDTTAWGADI

SEQ ID NO: 37 - protein, 19 aa, Unknown
  CDR stemming from rabbit antibody
GDDSSGYTDGGYAYWGLDI

SEQ ID NO: 38 - protein, 11 aa, Unknown
  CDR stemming from rabbit antibody
QASQSISSYLS

SEQ ID NO: 39 - protein, 11 aa, Unknown
  CDR stemming from rabbit antibody
QASQSIGSSLA

SEQ ID NO: 40 - protein, 13 aa, Unknown
  CDR stemming from rabbit antibody
QSSQSVWNNNRLA

SEQ ID NO: 41 - protein, 11 aa, Unknown
  CDR stemming from rabbit antibody
QASENINIWLS

SEQ ID NO: 42 - protein, 11 aa, Unknown
  CDR stemming from rabbit antibody
QASQSISSWLS

SEQ ID NO: 43 - protein, 11 aa, Unknown
  CDR stemming from rabbit antibody
QASEIIHSWLA

SEQ ID NO: 44 - protein, 11 aa, Unknown
  CDR stemming from rabbit antibody
QASQSINIWLS

SEQ ID NO: 45 - protein, 11 aa, Unknown
  CDR stemming from rabbit antibody
QADQSIYIWLS

SEQ ID NO: 46 - protein, 11 aa, Unknown
  CDR stemming from rabbit antibody
QASQNIRIWLS

SEQ ID NO: 47 - protein, 11 aa, Unknown
  CDR stemming from rabbit antibody
QASQSINIWCS

SEQ ID NO: 48 - protein, 11 aa, Unknown
  CDR stemming from rabbit antibody
QASQSINIWLS

SEQ ID NO: 49 - protein, 13 aa, Unknown
  CDR stemming from rabbit antibody
QASQSININNWLS

SEQ ID NO: 50 - protein, 7 aa, Unknown
  CDR stemming from rabbit antibody
KASTLAS

SEQ ID NO: 51 - protein, 7 aa, Unknown
  CDR stemming from rabbit antibody
TAANLAS

SEQ ID NO: 52 - protein, 7 aa, Unknown
  CDR stemming from rabbit antibody
YASTLAS

SEQ ID NO: 53 - protein, 7 aa, Unknown
  CDR stemming from rabbit antibody
QASKLAS

SEQ ID NO: 54 - protein, 7 aa, Unknown
  CDR stemming from rabbit antibody
QASTLAS

SEQ ID NO: 55 - protein, 7 aa, Unknown
  CDR stemming from rabbit antibody
LASTLAS

SEQ ID NO: 56 - protein, 7 aa, Unknown
  CDR stemming from rabbit antibody
KESTLAS

SEQ ID NO: 57 - protein, 7 aa, Unknown
  CDR stemming from rabbit antibody
KASTLES

SEQ ID NO: 58 - protein, 7 aa, Unknown
  CDR stemming from rabbit antibody
KASTLES

SEQ ID NO: 59 - protein, 7 aa, Unknown
  CDR stemming from rabbit antibody
RASTLAS

SEQ ID NO: 60 - protein, 7 aa, Unknown
  CDR stemming from rabbit antibody
KASTLAS

SEQ ID NO: 61 - protein, 14 aa, Unknown
  CDR stemming from rabbit antibody
QSNYGGSSSDYGNP

SEQ ID NO: 62 - protein, 10 aa, Unknown
  CDR stemming from rabbit antibody
QNFATSDTVT

SEQ ID NO: 63 - protein, 11 aa, Unknown
  CDR stemming from rabbit antibody
AGGYSSTSDNT

SEQ ID NO: 64 - protein, 12 aa, Unknown
  CDR stemming from rabbit antibody
QNNYSYNRYGAP

SEQ ID NO: 65 - protein, 12 aa, Unknown
  CDR stemming from rabbit antibody
QNNYGFRSYGGA

SEQ ID NO: 66 - protein, 12 aa, Unknown
  CDR stemming from rabbit antibody
QNVYLASTNGAN

SEQ ID NO: 67 - protein, 12 aa, Unknown
  CDR stemming from rabbit antibody
QNNYDSGNNGFP

SEQ ID NO: 68 - protein, 12 aa, Unknown
  CDR stemming from rabbit antibody
QNNAHYSTNGGT

SEQ ID NO: 69 - protein, 12 aa, Unknown
  CDR stemming from rabbit antibody
QNNAHYSTNGGT

SEQ ID NO: 70 - protein, 13 aa, Unknown
  CDR stemming from rabbit antibody
QANYAYSAGYGAA

SEQ ID NO: 71 - protein, 14 aa, Unknown
  CDR stemming from rabbit antibody
QNNYHYSSSTNGGT

SEQ ID NO: 72 - protein, 112 aa, Artificial Sequence
  recombinant scFv - VL sequence
EVVMAQTPASVEAAVGGTVTIKCQASQSISSYLSWYQQKPGQPPKLLIYKASTLASGVPSRFKGSRSGTEYTLTISDLECADAATYYCQSNYGGSSSDYGNPFGGGTEAVVK

SEQ ID NO: 73 - protein, 108 aa, Artificial Sequence
  recombinant scFv - VL sequence
AFELTQTPSSVEAAVGGTVTIKCQASQSIGSSLAWYQQKPGQRPKLLIYTAANLASGVPSRFRGSRSGAAFTLTISDLECADAATYYCQNFATSDTVTFGGGTEVVVT

SEQ ID NO: 74 - protein, 111 aa, Artificial Sequence
  recombinant scFv - VL sequence
AVVLTQTPSPVSAAVGGTVSISCQSSQSVWNNNRLAWFQQKSGQPPKLLIYYASTLASGVPSRFKGSGSGTEFTLTISDVQCDDAATYYCAGGYSSTSDNTFGGGTEVVVK

SEQ ID NO: 75 - protein, 110 aa, Artificial Sequence
  recombinant scFv - VL sequence
DIVMTQTPASVEATVGGTITINCQASENINIWLSWYQQKPGQPPKLLIYQASKLASGVPSRFKGSGSGTQFTLTISDLECADAATYYCQNNYSYNRYGAPFGGGTEVVVK

SEQ ID NO: 76 - protein, 110 aa, Artificial Sequence
  recombinant scFv - VL sequence
DVVMTQTPASVSEPVGGTVTIKCQASQSISSWLSWYQQKPGQPPKLLIYQASTLASGVPPRSSGSGSGTEYTLTISDLECADAATYFCQNNYGFRSYGGAFGGGTEVVVK

SEQ ID NO: 77 - protein, 110 aa, Artificial Sequence
  recombinant scFv - VL sequence
DVVMTQTPSSVSAAVGDTVTINCQASEIIHSWLAWYQQKPGQPPKLLIYLASTLASGVPSRFKGSGSGTQFTLTISDLECADAAIYYCQNVYLASTNGANFGGGTEVVVK

SEQ ID NO: 78 - protein, 110 aa, Artificial Sequence
  recombinant scFv - VL sequence
DVVMTQTPSSVSAAVGDTVTIKCQASQSINIWLSWYQQKSGQPPKLLVYKESTLASGVPSRFRGSGSGTQFTLTISDLECADAATYYCQNNYDSGNNGFPFGGGTEVVVK

SEQ ID NO: 79 - protein, 110 aa, Artificial Sequence
  recombinant scFv - VL sequence
DVVMTQTPSSVSAAVGDTVTINCQADQSIYIWLSWYQQKPGQPPKLLIYKASTLESGVPSRFKGSGSGTQFTLTISDLECADAATYYCQNNAHYSTNGGTFGGGTEVVVK

SEQ ID NO: 80 - protein, 110 aa, Artificial Sequence
  recombinant scFv - VL sequence
DVVMTQTPSSVSAAVGDTVTIKCQASQNIRIWLSWYQQKPGQPPKLLIYKASTLESGVPSRFKGSGSGTEFTLTISDLECADAATYYCQNNAHYSTNGGTFGGGTEVVVK

SEQ ID NO: 81 - protein, 111 aa, Artificial Sequence
  recombinant scFv - VL sequence
EVVMTQTPASVEAAVGGTVTIKCQASQSINIWCSWYQQKPGHPPKLLIYRASTLASGVSSRFKGSGSGTEFTLTISDLECADAATYYCQANYAYSAGYGAAFGGGTEVVVK

SEQ ID NO: 82 - protein, 113 aa, Artificial Sequence
  recombinant scFv - VL sequence
EIVMTQSPSTLSASVGDRVIITCQASQSISSYLSWYQQKPGKAPKLLIYKASTLASGVPSRFSGSGSGAEFTLTISSLQPDDFATYYCQSNYGGSSSDYGNPFGQGTKLTVLG

SEQ ID NO: 83 - protein, 109 aa, Artificial Sequence
  recombinant scFv - VL sequence
EIVMTQSPSTLSASVGDRVIITCQASQSIGSSLAWYQQKPGKAPKLLIYTAANLASGVPSRFSGSGSGAEFTLTISSLQPDDFATYYCQNFATSDTVTFGQGTKLTVLG

SEQ ID NO: 84 - protein, 112 aa, Artificial Sequence
  recombinant scFv - VL sequence
EIVMTQSPSTLSASVGDRVIITCQSSQSVWNNNRLAWYQQKPGKAPKLLIYYASTLASGVPSRFSGSGSGAEFTLTISSLQPDDFATYYCAGGYSSTSDNTFGQGTKLTVLG

SEQ ID NO: 85 - protein, 111 aa, Artificial Sequence
  recombinant scFv - VL sequence
EIVMTQSPSTLSASVGDRVIITCQASENINIWLSWYQQKPGKAPKLLIYQASKLASGVPSRFSGSGSGAEFTLTISSLQPDDFATYYCQNNYSYNRYGAPFGQGTKLTVLG

SEQ ID NO: 86 - protein, 111 aa, artificial sequence
  recombinant scFv - VL sequence
EIVMTQSPSTLSASVGDRVIITCQASQSISSWLSWYQQKPGKAPKLLIYQASTLASGVPSRFSGSGSGAEFTLTISSLQPDDFATYYCQNNYGFRSYGGAFGQGTKLTVLG

SEQ ID NO: 87 - protein, 111 aa, Artificial Sequence
  recombinant scFv - VL sequence
EIVMTQSPSTLSASVGDRVIITCQASEIIHSWLAWYQQKPGKAPKLLIYLASTLASGVPSRFSGSGSGAEFTLTISSLQPDDFATYYCQNVYLASTNGANFGQGTKLTVLG

SEQ ID NO: 88 - protein, 111 aa, Artificial Sequence
  recombinant scFv - VL sequence
EIVMTQSPSTLSASVGDRVIITCQASQSINIWLSWYQQKPGKAPKLLIYKESTLASGVPSRFSGSGSGAEFTLTISSLQPDDFATYYCQNNYDSGNNGFPFGQGTKLTVLG

SEQ ID NO: 89 - protein, 111 aa, Artificial Sequence
  recombinant scFv - VL sequence
EIVMTQSPSTLSASVGDRVIITCQADQSIYIWLSWYQQKPGKAPKLLIYKASTLESGVPSRFSGSGSGAEFTLTISSLQPDDFATYYCQNNAHYSTNGGTFGQGTKLTVLG

SEQ ID NO: 90 - protein, 111 aa, Artificial Sequence
  recombinant scFv - VL sequence
EIVMTQSPSTLSASVGDRVIITCQASQNIRIWLSWYQQKPGKAPKLLIYKASTLESGVPSRFSGSGSGAEFTLTISSLQPDDFATYYCQNNAHYSTNGGTFGQGTKLTVLG

SEQ ID NO: 91 - protein, 112 aa, Artificial Sequence
  recombinant scFv - VL sequence
EIVMTQSPSTLSASVGDRVIITCQASQSINIWCSWYQQKPGKAPKLLIYRASTLASGVPSRFSGSGSGAEFTLTISSLQPDDFATYYCQANYAYSAGYGAAFGQGTKLTVLG

SEQ ID NO: 92 - protein, 111 aa, Artificial Sequence
  recombinant scFv - VL sequence
EIVLTQSPSSLSASVGDRVTITCQASEIIHSWLAWYQQRPGKAPKLLISLASTLASGVPSRFSGSGSGTDFTFTISSLQPEDFAVYYCQNVYLASTNGANFGQGTKVEIKR

SEQ ID NO: 93 - protein, 113 aa, Artificial Sequence
  recombinant scFv - VL sequence
EIVMTQSPSTLSASVGDRVIITCQASQSISSYLSWYQQKPGKAPKLLIYKASTLASGVPSRFSGSGSGTEFTLTISSLQPDDFATYYCQSNYGGSSSDYGNPFGQGTKLTVLG

SEQ ID NO: 94 - protein, 109 aa, Artificial Sequence
  recombinant scFv - VL sequence
EIVMTQSPSTLSASVGDRVIIKCQASQSIGSSLAWYQQKPGKAPKLLIYTAANLASGVPSRFSGSGSGAEFTLTISSLQPDDFATYYCQNFATSDTVTFGQGTKLTVLG

SEQ ID NO: 95 - protein, 112 aa, Artificial Sequence
  recombinant scFv - VL sequence
EIVMTQSPSTLSASVGDRVIITCQSSQSVWNNNRLAWYQQKPGKAPKLLIYYASTLASGVPSRFSGSGSGTEFTLTISSLQPDDFATYYCAGGYSSTSDNTFGQGTKLTVLG

SEQ ID NO: 96 - protein, 111 aa, Artificial Sequence
  recombinant scFv - VL sequence
EIVMTQSPSTLSASVGDRVIITCQASENINIWLSWYQQKPGKAPKLLIYQASKLASGVPSRFSGSGSGTQFTLTISSLQPDDFATYYCQNNYSYNRYGAPFGQGTKLTVLG

SEQ ID NO: 97 - protein, 111 aa, Artificial Sequence
  recombinant scFv - VL sequence
EIVMTQSPSTLSASVGDRVIITCQASQSISSWLSWYQQKPGKAPKLLIYQASTLASGVPSRFSGSGSGTEFTLTISSLQPDDFATYYCQNNYGFRSYGGAFGQGTKLTVLG

SEQ ID NO: 98 - protein, 111 aa, Artificial Sequence
  recombinant scFv - VL sequence
EIVMTQSPSTLSASVGDRVIITCQASEIIHSWLAWYQQKPGKAPKLLIYLASTLASGVPSRFSGSGSGTQFTLTISSLQPDDFATYYCQNVYLASTNGANFGQGTKLTVLG

SEQ ID NO: 99 - protein, 111 aa, Artificial Sequence
  recombinant scFv - VL sequence
EIVMTQSPSTLSASVGDRVIITCQASQSINIWLSWYQQKPGKAPKLLIYKESTLASGVPSRFSGSGSGTEFTLTISSLQPDDFATYYCQNNYDSGNNGFPFGQGTKLTVLG

SEQ ID NO: 100 - protein, 111 aa, Artificial Sequence
  recombinant scFv - VL sequence
EIVMTQSPSTLSASVGDRVIITCQADQSIYIWLSWYQQKPGKAPKLLIYKASTLESGVPSRFSGSGSGTQFTLTISSLQPDDFATYYCQNNAHYSTNGGTFGQGTKLTVLG

SEQ ID NO: 101 - protein, 111 aa, Artificial Sequence
  recombinant scFv - VL sequence
EIVMTQSPSTLSASVGDRVIITCQASQNIRIWLSWYQQKPGKAPKLLIYKASTLESGVPSRFSGSGSGTEFTLTISSLQPDDFATYYCQNNAHYSTNGGTFGQGTKLTVLG

SEQ ID NO: 102 - protein, 112 aa, Artificial Sequence
  recombinant scFv - VL sequence
EIVMTQSPSTLSASVGDRVIITCQASQSINIWLSWYQQKPGKAPKLLIYRASTLASGVPSRFSGSGSGTEFTLTISSLQPDDFATYYCQANYAYSAGYGAAFGQGTKLTVLG

SEQ ID NO: 103 - protein, 111 aa, Artificial Sequence
  recombinant scFv - VL sequence
EIVMTQSPSSLSASVGDRVTITCQASEIIHSWLAWYQQRPGKAPKLLISLASTLASGVPSRFSGSGSGTQFTFTISSLQPEDFAVYYCQNVYLASTNGANFGQGTKVEIKR

SEQ ID NO: 104 - protein, 111 aa, Artificial Sequence
  recombinant scFv - VL sequence
DIVMTQSPSTLSASVGDRVIITCQASEIIHSWLAWYQQKPGKAPKLLIYLASTLASGVPSRFSGSGSGAEFTLTISSLQPDDFATYYCQNVYLASTNGANFGQGTKLTVLG

SEQ ID NO: 105 - protein, 111 aa, Artificial Sequence
  recombinant scFv - VL sequence
EVVMTQSPSTLSASVGDRVIITCQASEIIHSWLAWYQQKPGKAPKLLIYLASTLASGVPSRFSGSGSGAEFTLTISSLQPDDFATYYCQNVYLASTNGANFGQGTKLTVLG

SEQ ID NO: 106 - protein, 112 aa, Artificial Sequence
  recombinant scFv - VL sequence
EIVMTQSPSTLSASVGDRVIITCQASQSINIWLSWYQQKPGKAPKLLIYRASTLASGVPSRFSGSGSGAEFTLTISSLQPDDFATYYCQANYAYSAGYGAAFGQGTKLTVLG

SEQ ID NO: 107 - protein, 128 aa, Artificial Sequence
  recombinant scFv - VH sequence
QSLEESGGDLVKPGASLTLTCTASGFPFSSGYWVCWVRQAPGKGLEWIACIYAGSSGSTYYASWAKGRFTISKTSSTTVTLQMTSLTAADTATYFCARGNNYYIYTDGGYAYAGLELWGPGILVTVSS

SEQ ID NO: 108 - protein, 128 aa, Artificial Sequence
  recombinant scFv - VH sequence
QSLEESGGDLVKPGASLTLTCTASGFSFSSGYWICWVRQAPGKGLEWIACIYAGSSGSTYYASWAKGRFTISKTSSTTVTLQMTSLTAADTATYFCARGNNYYIYTDGGYAYAGLELWGPGILVTVSS

SEQ ID NO: 109 - protein, 117 aa, Artificial Sequence
  recombinant scFv - VH sequence
QSLEESGGDLVQPGASLTLTCKVSGFSLNTNYWMCWVRQAPGKGLEWIGCMYTGSYNRAYYASWAKGRFTSSKTSSTTVTLEMTSLTAADTATYFCAKGSNWYSDLWGPGTLVTVSS

SEQ ID NO: 110 - protein, 124 aa, Artificial Sequence
  recombinant scFv - VH sequence
QERLVESGGGLVQPEGSLTLTCKASGFSFSRSYYIYWVRQAPGKGLEWIACIDAGSSGILVYANWAKGRFTISKTSSTTVTLQMTSLTAADTATYFCARGDASYGVDSFMLPLWGPGTLVTVSS

SEQ ID NO: 111 - protein, 119 aa, Artificial Sequence
  recombinant scFv - VH sequence
QSLEESGGGLVQPEGSLTLTCKASGFSFTTTDYMCWVRQAPGKGLEWIGCILAGDGSTYYANWAKGRFTGSKTSSTTVDLKMTGLTAADTATYFCARSDPASSWSFALWGPGTLVTVSS

SEQ ID NO: 112 - protein, 117 aa, Artificial Sequence
  recombinant scFv - VH sequence
QSLEESGGRLVTPGTPLTLTCTASGIDFSGAYYMGWVRQAPGKGLEWIGYIDYDGDRYYASWAKGRFTISKTSTTVDLKITSPTTEDTATYFCARSDYSSGWGTDIWGPGTLVTVSL

SEQ ID NO: 113 - protein, 117 aa, Artificial Sequence
  recombinant scFv - VH sequence
QSVEESGGRLVTPGTPLTLTCTASGFSLTDYYYMTWVRLAPGKGLEYIGFIDPDDDPYYATWAKGRFTISRTSTTVNLKMTSPTTEDTATYFCAGGDHNSGWGLDIWGPGTLVTVSL

SEQ ID NO: 114 - protein, 116 aa, Artificial Sequence
  recombinant scFv - VH sequence
QSLEESGGRLVTPGTPLTLTCTASGFSLSYYYMSWVRQAPGKGLEWIGIIGPGDYTDYASWAKGRFTISKTSTTVDLKITSPTTEDTATYFCGRGDDNSGWGEDIWGPGTLVTVSL

SEQ ID NO: 115 - protein, 116 aa, Artificial Sequence
  recombinant scFv - VH sequence
QSVEESGGRLVTPGAPLTLTCSVSGFSLSDYYMCWVRQAPGKGLQWIGCLDYFGSTDDASWAKGRFTISKTSTAVDLKITSPTTEDTATYFCARTDDSRGWGLNIWGPGTLVTVSL

SEQ ID NO: 116 - protein, 116 aa, Artificial Sequence
  recombinant scFv - VH sequence
QSLEESGGRLVTPGTPLTLTCTASGFSLSSYYMCWVRQAPGKGLEWIGCLDYVGDTDYASWAKGRFTISKASTTVDLKITSLTTEDTATYFCARTDDSRGWGLNIWGPGTLVTVSL

SEQ ID NO: 117 - protein, 118 aa, Artificial Sequence
  recombinant scFv - VH sequence
QSVEESGGRLVTPGTPLTLTCTVSGFSLNTYYMNWVRQAPGKGLEWIGIIAPDDTTYYASWAKSRSTITRDTNENTVTLKMTSLTTEDTATYFCARSGDTTAWGADIWGPGTLVTVSL

SEQ ID NO: 118 - protein, 130 aa, Artificial Sequence
  recombinant scFv - VH sequence
EVQLVESGGGLVQPGGSLRLSCAASGFPFSSGYWVCWVRQAPGKGLEWVSCIYAGSSGSTYYASWAKGRFTISRDNSKNTLYLQMNSLRAEDTAVYYCAKGNNYYIYTDGGYAYAGLELWGQGTLVTVSS

SEQ ID NO: 119 - protein, 130 aa, Artificial Sequence
  recombinant scFv - VH sequence
EVQLVESGGGLVQPGGSLRLSCAASGFSFSSGYWICWVRQAPGKGLEWVSCIYAGSSGSTYYASWAKGRFTISRDNSKNTLYLQMNSLRAEDTAVYYCAKGNNYYIYTDGGYAYAGLELWGQGTLVTVSS

SEQ ID NO: 120 - protein, 119 aa, Artificial Sequence
  recombinant scFv - VH sequence
EVQLVESGGGLVQPGGSLRLSCAASGFSLNTNYWMCWVRQAPGKGLEWVSCMYTGSYNRAYYASWAKGRFTISRDNSKNTLYLQMNSLRAEDTAVYYCAKGSNWYSDLWGQGTLVTVSS

SEQ ID NO: 121 - protein, 125 aa, Artificial Sequence
  recombinant scFv - VH sequence
EVQLVESGGGLVQPGGSLRLSCAASGFSFSRSYYIYWVRQAPGKGLEWVSCIDAGSSGILVYANWAKGRFTISRDNSKNTLYLQMNSLRAEDTAVYYCAKGDASYGVDSFMLPLWGQGTLVTVSS

SEQ ID NO: 122 - protein, 121 aa, Artificial Sequence
  recombinant scFv - VH sequence
EVQLVESGGGLVQPGGSLRLSCAASGFSFTTTDYMCWVRQAPGKGLEWVSCILAGDGSTYYANWAKGRFTISRDNSKNTLYLQMNSLRAEDTAVYYCAKSDPASSWSFALWGQGTLVTVSS

SEQ ID NO: 123 - protein, 120 aa, Artificial Sequence
  recombinant scFv - VH sequence
EVQLVESGGGLVQPGGSLRLSCAASGIDFSGAYYMGWVRQAPGKGLEWVSYIDYDGDRYYASWAKGRFTISRDNSKNTLYLQMNSLRAEDTAVYYCAKSDYSSGWGTDIWGQGTLVTVSS

SEQ ID NO: 124 - protein, 120 aa, Artificial Sequence
  recombinant scFv - VH sequence
EVQLVESGGGLVQPGGSLRLSCAASGFSLTDYYYMTWVRQAPGKGLEWVSFIDPDDDPYYATWAKGRFTISRDNSKNTLYLQMNSLRAEDTAVYYCAKGDHNSGWGLDIWGQGTLVTVSS

SEQ ID NO: 125 - protein, 119 aa, Artificial Sequence
  recombinant scFv - VH sequence
EVQLVESGGGLVQPGGSLRLSCAASGFSLSYYYMSWVRQAPGKGLEWVSIIGPGDYTDYASWAKGRFTISRDNSKNTLYLQMNSLRAEDTAVYYCAKGDDNSGWGEDIWGQGTLVTVSS

SEQ ID NO: 126 - protein, 119 aa, Artificial Sequence
  recombinant scFv - VH sequence
EVQLVESGGGLVQPGGSLRLSCAASGFSLSDYYMCWVRQAPGKGLEWVSCLDYFGSTDDASWAKGRFTISRDNSKNTLYLQMNSLRAEDTAVYYCAKTDDSRGWGLNIWGQGTLVTVSS

SEQ ID NO: 127 - protein, 119 aa, Artificial Sequence
  recombinant scFv - VH sequence
EVQLVESGGGLVQPGGSLRLSCAASGFSLSSYYMCWVRQAPGKGLEWVSCLDYVGDTDYASWAKGRFTISRDNSKNTLYLQMNSLRAEDTAVYYCAKTDDSRGWGLNIWGQGTLVTVSS

SEQ ID NO: 128 - protein, 119 aa, Artificial Sequence
  recombinant scFv - VH sequence
EVQLVESGGGLVQPGGSLRLSCAASGFSLNTYYMNWVRQAPGKGLEWVSIIAPDDTTYYASWAKSRFTISRDNSKNTLYLQMNSLRAEDTAVYYCAKSGDTTAWGADIWGQGTLVTVSS

SEQ ID NO: 129 - protein, 120 aa, Artificial Sequence
  recombinant scFv - VH sequence
QVQLVQTGGGLVQPGGSLRLSCAASGFSLTDYYYMTWVRQAPGKGLEWVSFIDPDDDPYYATWAKGRFTISRDNSKNTVYLQMNSLRAEDTALYYCAKGDHNSGWGLDIWGQGTLVTVSS

SEQ ID NO: 130 - protein, 130 aa, Artificial Sequence
  recombinant scFv - VH sequence
EVQLVESGGGLVQPGGSLRLSCTASGFPFSSGYWVCWVRQAPGKGLEWVGCIYAGSSGSTYYASWAKGRFTISKDTSKNTVYLQMNSLRAEDTAVYYCARGNNYYIYTDGGYAYAGLELWGQGTLVTVSS

SEQ ID NO: 131 - protein, 130 aa, Artificial Sequence
  recombinant scFv - VH sequence
EVQLVESGGGLVQPGGSLRLSCTASGFSFSSGYWICWVRQAPGKGLEWVGCIYAGSSGSTYYASWAKGRFTISKDTSKNTVYLQMNSLRAEDTAVYYCARGNNYYIYTDGGYAYAGLELWGQGTLVTVSS

SEQ ID NO: 132 - protein, 119 aa, Artificial Sequence
  recombinant scFv - VH sequence
EVQLVESGGGLVQPGGSLRLSCKVSGFSLNTNYWMCWVRQAPGKGLEWVGCMYTGSYNRAYYASWAKGRFTSSKDTSKNTVYLQMNSLRAEDTAVYYCAKGSNWYSDLWGQGTLVTVSS

SEQ ID NO: 133 - protein, 125 aa, Artificial Sequence
  recombinant scFv - VH sequence
EVQLVESGGGLVQPGGSLRLSCKASGFSFSRSYYIYWVRQAPGKGLEWVGCIDAGSSGILVYANWAKGRFTISKDTSKNTVYLQMNSLRAEDTAVYYCARGDASYGVDSFMLPLWGQGTLVTVSS

SEQ ID NO: 134 - protein, 121 aa, Artificial Sequence
  recombinant scFv - VH sequence
EVQLVESGGGLVQPGGSLRLSCKASGFSFTTTDYMCWVRQAPGKGLEWVGCILAGDGSTYYANWAKGRFTGSKDTSKNTVYLQMNSLRAEDTAVYYCARSDPASSWSFALWGQGTLVTVSS

SEQ ID NO: 135 - protein, 120 aa, Artificial Sequence
  recombinant scFv - VH sequence
EVQLVESGGGLVQPGGSLRLSCTASGIDFSGAYYMGWVRQAPGKGLEWVGYIDYDGDRYYASWAKGRFTISKDTSKNTVYLQMNSLRAEDTAVYYCARSDYSSGWGTDIWGQGTLVTVSS

SEQ ID NO: 136 - protein, 120 aa, Artificial Sequence
  recombinant scFv - VH sequence
EVQLVESGGGLVQPGGSLRLSCTASGFSLTDYYYMTWVRQAPGKGLEWVGFIDPDDDPYYATWAKGRFTISRDTSKNTVYLQMNSLRAEDTAVYYCAGGDHNSGWGLDIWGQGTLVTVSS

SEQ ID NO: 137 - protein, 119 aa, Artificial Sequence
  recombinant scFv - VH sequence
EVQLVESGGGLVQPGGSLRLSCTASGFSLSYYYMSWVRQAPGKGLEWVGIIGPGDYTDYASWAKGRFTISKDTSKNTVYLQMNSLRAEDTAVYYCARGDDNSGWGEDIWGQGTLVTVSS

SEQ ID NO: 138 - protein, 119 aa, Artificial Sequence
  recombinant scFv - VH sequence
EVQLVESGGGLVQPGGSLRLSCSVSGFSLSDYYMCWVRQAPGKGLEWVGCLDYFGSTDDASWAKGRFTISKDTSKNTVYLQMNSLRAEDTAVYYCARTDDSRGWGLNIWGQGTLVTVSS

SEQ ID NO: 139 - protein, 119 aa, Artificial Sequence
  recombinant scFv - VH sequence
EVQLVESGGGLVQPGGSLRLSCTASGFSLSSYYMCWVRQAPGKGLEWVGCLDYVGDTDYASWAKGRFTISKDASKNTVYLQMNSLRAEDTAVYYCARTDDSRGWGLNIWGQGTLVTVSS

SEQ ID NO: 140 - protein, 119 aa, Artificial Sequence
  recombinant scFv - VH sequence
EVQLVESGGGLVQPGGSLRLSCTASGFSLSSYYMSWVRQAPGKGLEWVGILDYVGDTDYASWAKGRFTISKDASKNTVYLQMNSLRAEDTAVYYCARTDDSRGWGLNIWGQGTLVTVSS

SEQ ID NO: 141 - protein, 119 aa, Artificial Sequence
  recombinant scFv - VH sequence
EVQLVESGGGLVQPGGSLRLSCTVSGFSLNTYYMNWVRQAPGKGLEWVGIIAPDDTTYYASWAKSRSTISRDTSKNTVYLQMNSLRAEDTAVYYCARSGDTTAWGADIWGQGTLVTVSS

SEQ ID NO: 142 - protein, 120 aa, Artificial Sequence
  recombinant scFv - VH sequence
QVQLVQTGGGLVQPGGSLRLSCTASGFSLTDYYYMTWVRQAPGKGLEWVGFIDPDDDPYYATWAKGRFTISRDTSKNTVYLQMNSLRAEDTALYYCAGGDHNSGWGLDIWGQGTLVTVSS

SEQ ID NO: 143 - protein, 119 aa, Artificial Sequence
  recombinant scFv - VH sequence
EVQLVESGGGSVQPGGSLRLSCAASGFSLSDYYMCWVRQAPGKGLEWVSCLDYFGSTDDASWAKGRFTISRDNSKNTLYLQMNSLRAEDTATYYCAKTDDSRGWGLNIWGQGTTVTVSS

SEQ ID NO: 144 - protein, 120 aa, Artificial Sequence
  recombinant scFv - VH sequence
EVQLVESGGGSVQPGGSLRLSCTASGFSLTDYYYMTWVRQAPGKGLEWVGFIDPDDDPYYATWAKGRFTISRDTSKNTVYLQMNSLRAEDTATYYCAGGDHNSGWGLDIWGQGTTVTVSS

SEQ ID NO: 145 - protein, 119 aa, Artificial Sequence
  recombinant scFv - VH sequence
EVQLVESGGGSVQPGGSLRLSCTVSGFSLNTYYMNWVRQAPGKGLEWVGIIAPDDTTYYASWAKSRSTISRDTSKNTVYLQMNSLRAEDTATYYCARSGDTTAWGADIWGQGTTVTVSS

SEQ ID NO: 146 - protein, 120 aa, Artificial Sequence
  recombinant scFv - VH sequence
QVQLVQTGGGSVQPGGSLRLSCTASGFSLTDYYYMTWVRQAPGKGLEWVGFIDPDDDPYYATWAKGRFTISRDTSKNTVYLQMNSLRAEDTATYYCAGGDHNSGWGLDIWGQGTTVTVSS

SEQ ID NO: 147 - protein, 119 aa, Artificial Sequence
  recombinant scFv - VH sequence
VQLVESGGGLVQPGGSLRLSCTASGFSLTDYYYMTWVRQAPGKGLEWVGFIDPDDDPYYATWAKGRFTISRDTSKNTVYLQMNSLRAEDTAVYYCAGGDHNSGWGLDIWGQGTLVTVSS

SEQ ID NO: 148 - protein, 120 aa, Artificial Sequence
  recombinant scFv - VH sequence
EQQLVESGGGLVQPGGSLRLSCTASGFSLTDYYYMTWVRQAPGKGLEWVGFIDPDDDPYYATWAKGRFTISRDTSKNTVYLQMNSLRAEDTAVYYCAGGDHNSGWGLDIWGQGTLVTVSS

SEQ ID NO: 149 - protein, 120 aa, Artificial Sequence
  recombinant scFv - VH sequence
EVQLVESGGGLVQPGGSLRLSCTASGFSLTDYYYMTWVRLAPGKGLEWVGFIDPDDDPYYATWAKGRFTISRDTSKNTVYLQMNSLRAEDTAVYYCAGGDHNSGWGLDIWGQGTLVTVSS

SEQ ID NO: 150 - protein, 120 aa, Artificial Sequence
  recombinant scFv - VH sequence
EVQLVESGGGLVQPGGSLRLSCTASGFSLTDYYYMTWVRQAPGKGLEYVGFIDPDDDPYYATWAKGRFTISRDTSKNTVYLQMNSLRAEDTAVYYCAGGDHNSGWGLDIWGQGTLVTVSS

SEQ ID NO: 151 - protein, 120 aa, Artificial Sequence
  recombinant scFv - VH sequence
EVQLVESGGGLVQPGGSLRLSCTASGFSLTDYYYMTWVRQAPGKGLEWIGFIDPDDDPYYATWAKGRFTISRDTSKNTVYLQMNSLRAEDTAVYYCAGGDHNSGWGLDIWGQGTLVTVSS

SEQ ID NO: 152 - protein, 120 aa, Artificial Sequence
  recombinant scFv - VH sequence
EVQLVESGGGLVQPGGSLRLSCTASGFSLTDYYYMTWVRQAPGKGLEWVGFIDPDDDPYYATWAKGRFTISRATSKNTVYLQMNSLRAEDTAVYYCAGGDHNSGWGLDIWGQGTLVTVSS

SEQ ID NO: 153 - protein, 120 aa, Artificial Sequence
  recombinant scFv - VH sequence
EVQLVESGGGLVQPGGSLRLSCTASGFSLTDYYYMTWVRQAPGKGLEWVGFIDPDDDPYYATWAKGRFTISRDTSKATVYLQMNSLRAEDTAVYYCAGGDHNSGWGLDIWGQGTLVTVSS

SEQ ID NO: 154 - protein, 120 aa, Artificial Sequence
  recombinant scFv - VH sequence
EVQLVESGGGLVQPGGSLRLSCTASGFSLTDYYYMTWVRQAPGKGLEWVGFIDPDDDPYYATWAKGRFTISRDTSKNTVYLQMNSLRAEDTAVYFCAGGDHNSGWGLDIWGQGTLVTVSS

SEQ ID NO: 155 - protein, 119 aa, Artificial Sequence
  recombinant scFv - VH sequence
EVQLVESGGGLVQPGGSLRLSCTASGFSLTDYYYMTWVRQAPGKGLEWVGFIDPDDDPYYATWAKGRFTISRTSKNTVYLQMNSLRAEDTAVYYCAGGDHNSGWGLDIWGQGTLVTVSS

SEQ ID NO: 156 - protein, 119 aa, Artificial Sequence
  recombinant scFv - VH sequence
EVQLVESGGGLVQPGGSLRLSCTASGFSLTDYYYMTWVRQAPGKGLEWVGFIDPDDDPYYATWAKGRFTISRDTSKTVYLQMNSLRAEDTAVYYCAGGDHNSGWGLDIWGQGTLVTVSS

SEQ ID NO: 157 - protein, 120 aa, Artificial Sequence
  recombinant scFv - VH sequence
EVQLVESGGGLVQPGGSLRLSCTASGFSLTDYYYMTWVRQAPGKGLEWVGFIDPDDDPYYATWAKGRFTISRDNSKNTVYLQMNSLRAEDTAVYYCAGGDHNSGWGLDIWGQGTLVTVSS

SEQ ID NO: 158 - protein, 120 aa, Artificial Sequence
  recombinant scFv - VH sequence
EVQLVESGGGLVQPGGSLRLSCTASGFSLTDYYYMTWVRQAPGKGLEWVGFIDPDDDPYYATWAKGRFTISRDTSKNTLYLQMNSLRAEDTAVYYCAGGDHNSGWGLDIWGQGTLVTVSS

SEQ ID NO: 159 - protein, 120 aa, Artificial Sequence
  recombinant scFv - VH sequence
EVQLVESGGGLVQPGGSLRLSCTASGFSLTDYYYMTWVRQAPGKGLEWVGFIDPDDDPYYATWAKGRFTISRDTSKNTAYLQMNSLRAEDTAVYYCAGGDHNSGWGLDIWGQGTLVTVSS

SEQ ID NO: 160 - protein, 120 aa, Artificial Sequence
  recombinant scFv - VH sequence
EVQLVESGGGSVQPGGSLRLSCTASGFSLTDYYYMTWVRQAPGKGLEWVGFIDPDDDPYYATWAKGRFTISRDNSKNTVYLQMNSLRAEDTATYYCAGGDHNSGWGLDIWGQGTTVTVSS

SEQ ID NO: 161 - protein, 120 aa, Artificial Sequence
  recombinant scFv - VH sequence
EVQLVESGGGSVQPGGSLRLSCTASGFSLTDYYYMTWVRQAPGKGLEWVGFIDPDDDPYYATWAKGRFTISRDTSKNTLYLQMNSLRAEDTATYYCAGGDHNSGWGLDIWGQGTTVTVSS

SEQ ID NO: 162 - protein, 120 aa, Artificial Sequence
  recombinant scFv - VH sequence
EVQLVESGGGSVQPGGSLRLSCTASGFSLTDYYYMTWVRQAPGKGLEWVGFIDPDDDPYYATWAKGRFTISRDTSKNTAYLQMNSLRAEDTATYYCAGGDHNSGWGLDIWGQGTTVTVSS

SEQ ID NO: 163 - protein, 120 aa, Artificial Sequence
  recombinant scFv - VH sequence
EVQLVESGGGLVQPGGSLRLSCTASGFSLTDYYYMTWVRQAPGKGLEWVGFIDPDDDPYYATWAKGRFTISRDNSKNTAYLQMNSLRAEDTAVYYCAGGDHNSGWGLDIWGQGTLVTVSS

SEQ ID NO: 164 - protein, 120 aa, Artificial Sequence
  recombinant scFv - VH sequence
EVQLVESGGGLVQPGGSLRLSCTASGFSLTDYYYMTWVRQAPGKGLEWVGFIDPDDDPYYATWAKGRFTISRDNSKNTLYLQMNSLRAEDTAVYYCAGGDHNSGWGLDIWGQGTLVTVSS

SEQ ID NO: 165 - protein, 120 aa, Artificial Sequence
  recombinant scFv - VH sequence
EVQLVESGGGSVQPGGSLRLSCTASGFSLTDYYYMTWVRQAPGKGLEWVGFIDPDDDPYYATWAKGRFTISRDNSKNTAYLQMNSLRAEDTATYYCAGGDHNSGWGLDIWGQGTTVTVSS

SEQ ID NO: 166 - protein, 120 aa, Artificial Sequence
  recombinant scFv - VH sequence
EVQLVESGGGSVQPGGSLRLSCTASGFSLTDYYYMTWVRQAPGKGLEWVGFIDPDDDPYYATWAKGRFTISRDNSKNTLYLQMNSLRAEDTATYYCAGGDHNSGWGLDIWGQGTTVTVSS

SEQ ID NO: 167 - protein, 381 aa, Artificial Sequence
  recombinant scFv - VL acceptor sequence
  CDR (24)..(123): At least 3 and up to 50 amino acids can be present
  CDR (139)..(238): At least 3 and up to 50 amino acids can be present
  CDR (271)..(370): At least 3 and up to 50 amino acids can be present
EIVMTQSPSTLSASVGDRVIITCXXXXXXXXXXXXXXXXXXXXXXXXXXXXXXXXXXXXXXXXXXXXXXXXXXXXXXXXXXXXXXXXXXXXXXXXXXXXXXXXXXXXXXXXXXXXXXXXXXXXWYQQKPGKAPKLLIYXXXXXXXXXXXXXXXXXXXXXXXXXXXXXXXXXXXXXXXXXXXXXXXXXXXXXXXXXXXXXXXXXXXXXXXXXXXXXXXXXXXXXXXXXXXXXXXXXXXXGVPSRFSGSGSGAEFTLTISSLQPDDFATYYCXXXXXXXXXXXXXXXXXXXXXXXXXXXXXXXXXXXXXXXXXXXXXXXXXXXXXXXXXXXXXXXXXXXXXXXXXXXXXXXXXXXXXXXXXXXXXXXXXXXXFGQGTKLTVLG

SEQ ID NO: 168 - protein, 381 aa, Artificial Sequence; identical to SEQ ID NO: 167
  recombinant scFv - VL acceptor sequence
  CDR (24)..(123): At least 3 and up to 50 amino acids can be present
  CDR (139)..(238): At least 3 and up to 50 amino acids can be present
  CDR (271)..(370): At least 3 and up to 50 amino acids can be present

SEQ ID NO: 169 - protein, 382 aa, Artificial Sequence
  recombinant scFv - VH acceptor sequence
  CDR (26)..(125): At least 3 and up to 50 amino acids can be present.
  CDR (140)..(239): At least 3 and up to 50 amino acids can be present.
  CDR (272)..(371): At least 3 and up to 50 amino acids can be present.
EVQLVESGGGLVQPGGSLRLSCAASXXXXXXXXXXXXXXXXXXXXXXXXXXXXXXXXXXXXXXXXXXXXXXXXXXXXXXXXXXXXXXXXXXXXXXXXXXXXXXXXXXXXXXXXXXXXXXXXXXXXWVRQAPGKGLEWVSXXXXXXXXXXXXXXXXXXXXXXXXXXXXXXXXXXXXXXXXXXXXXXXXXXXXXXXXXXXXXXXXXXXXXXXXXXXXXXXXXXXXXXXXXXXXXXXXXXXXRFTISRDNSKNTLYLQMNSLRAEDTAVYYCAKXXXXXXXXXXXXXXXXXXXXXXXXXXXXXXXXXXXXXXXXXXXXXXXXXXXXXXXXXXXXXXXXXXXXXXXXXXXXXXXXXXXXXXXXXXXXXXXXXXXXWGQGTLVTVSS

SEQ ID NO: 170 - protein, 381 aa, Artificial Sequence
  recombinant scFv - VH acceptor sequence
  CDR (26)..(125): At least 3 and up to 50 amino acids can be present.
  CDR (140)..(239): At least 3 and up to 50 amino acids can be present.
  CDR (272)..(371): At least 3 and up to 50 amino acids can be present.
EVQLVESGGGLVQPGGSLRLSCTASXXXXXXXXXXXXXXXXXXXXXXXXXXXXXXXXXXXXXXXXXXXXXXXXXXXXXXXXXXXXXXXXXXXXXXXXXXXXXXXXXXXXXXXXXXXXXXXXXXXXWVRQAPGKGLEWVGXXXXXXXXXXXXXXXXXXXXXXXXXXXXXXXXXXXXXXXXXXXXXXXXXXXXXXXXXXXXXXXXXXXXXXXXXXXXXXXXXXXXXXXXXXXXXXXXXXXXRFTISRDTSKNTVYLQMNSLRAEDTAVYYCARXXXXXXXXXXXXXXXXXXXXXXXXXXXXXXXXXXXXXXXXXXXXXXXXXXXXXXXXXXXXXXXXXXXXXXXXXXXXXXXXXXXXXXXXXXXXXXXXXXXXWGQGTLVTVS

SEQ ID NO: 171 - protein, 382 aa, Artificial Sequence
  recombinant scFv - VH acceptor sequence
  CDR (26)..(125): At least 3 and up to 50 amino acids can be present.
  CDR (140)..(239): At least 3 and up to 50 amino acids can be present.
  CDR (272)..(371): At least 3 and up to 50 amino acids can be present.
EVQLVESGGGLVQPGGSLRLSCTVSXXXXXXXXXXXXXXXXXXXXXXXXXXXXXXXXXXXXXXXXXXXXXXXXXXXXXXXXXXXXXXXXXXXXXXXXXXXXXXXXXXXXXXXXXXXXXXXXXXXXWVRQAPGKGLEWVGXXXXXXXXXXXXXXXXXXXXXXXXXXXXXXXXXXXXXXXXXXXXXXXXXXXXXXXXXXXXXXXXXXXXXXXXXXXXXXXXXXXXXXXXXXXXXXXXXXXXRFTISKDTSKNTVYLQMNSLRAEDTAVYYCARXXXXXXXXXXXXXXXXXXXXXXXXXXXXXXXXXXXXXXXXXXXXXXXXXXXXXXXXXXXXXXXXXXXXXXXXXXXXXXXXXXXXXXXXXXXXXXXXXXXXWGQGTLVTVSS

SEQ ID NO: 172 - protein, 783 aa, Artificial Sequence
  recombinant scFv - acceptor sequence
  CDR (24)..(123): At least 3 and up to 50 amino acids can be present.
  CDR (139)..(238): At least 3 and up to 50 amino acids can be present.
  CDR (271)..(370): At least 3 and up to 50 amino acids can be present.
  CDR (427)..(526): At least 3 and up to 50 amino acids can be present.
  CDR (541)..(640): At least 3 and up to 50 amino acids can be present.
  CDR (673)..(772): At least 3 and up to 50 amino acids can be present.
EIVMTQSPSTLSASVGDRVIITCXXXXXXXXXXXXXXXXXXXXXXXXXXXXXXXXXXXXXXXXXXXXXXXXXXXXXXXXXXXXXXXXXXXXXXXXXXXXXXXXXXXXXXXXXXXXXXXXXXXXWYQQKPGKAPKLLIYXXXXXXXXXXXXXXXXXXXXXXXXXXXXXXXXXXXXXXXXXXXXXXXXXXXXXXXXXXXXXXXXXXXXXXXXXXXXXXXXXXXXXXXXXXXXXXXXXXXXGVPSRFSGSGSGAEFTLTISSLQPDDFATYYCXXXXXXXXXXXXXXXXXXXXXXXXXXXXXXXXXXXXXXXXXXXXXXXXXXXXXXXXXXXXXXXXXXXXXXXXXXXXXXXXXXXXXXXXXXXXXXXXXXXXFGQGTKLTVLGGGGGSGGGGSGGGGSGGGGSEVQLVESGGGLVQPGGSLRLSCAASXXXXXXXXXXXXXXXXXXXXXXXXXXXXXXXXXXXXXXXXXXXXXXXXXXXXXXXXXXXXXXXXXXXXXXXXXXXXXXXXXXXXXXXXXXXXXXXXXXXXWVRQAPGKGLEWVSXXXXXXXXXXXXXXXXXXXXXXXXXXXXXXXXXXXXXXXXXXXXXXXXXXXXXXXXXXXXXXXXXXXXXXXXXXXXXXXXXXXXXXXXXXXXXXXXXXXXRFTISRDNSKNTLYLQMNSLRAEDTAVYYCAKXXXXXXXXXXXXXXXXXXXXXXXXXXXXXXXXXXXXXXXXXXXXXXXXXXXXXXXXXXXXXXXXXXXXXXXXXXXXXXXXXXXXXXXXXXXXXXXXXXXXWGQGTLVTVSS

SEQ ID NO: 173 - protein, 783 aa, Artificial Sequence
  recombinant scFv - acceptor sequence
  CDR (24)..(123): At least 3 and up to 50 amino acids can be present.
  CDR (139)..(238): At least 3 and up to 50 amino acids can be present.
  CDR (271)..(370): At least 3 and up to 50 amino acids can be present.
  CDR (427)..(526): At least 3 and up to 50 amino acids can be present.
  CDR (541)..(640): At least 3 and up to 50 amino acids can be present.
  CDR (673)..(772): At least 3 and up to 50 amino acids can be present.
EIVMTQSPSTLSASVGDRVIITCXXXXXXXXXXXXXXXXXXXXXXXXXXXXXXXXXXXXXXXXXXXXXXXXXXXXXXXXXXXXXXXXXXXXXXXXXXXXXXXXXXXXXXXXXXXXXXXXXXXXWYQQKPGKAPKLLIYXXXXXXXXXXXXXXXXXXXXXXXXXXXXXXXXXXXXXXXXXXXXXXXXXXXXXXXXXXXXXXXXXXXXXXXXXXXXXXXXXXXXXXXXXXXXXXXXXXXXGVPSRFSGSGSGTEFTLTISSLQPDDFATYYCXXXXXXXXXXXXXXXXXXXXXXXXXXXXXXXXXXXXXXXXXXXXXXXXXXXXXXXXXXXXXXXXXXXXXXXXXXXXXXXXXXXXXXXXXXXXXXXXXXXXFGQGTKLTVLGGGGGSGGGGSGGGGSGGGGSEVQLVESGGGLVQPGGSLRLSCTASXXXXXXXXXXXXXXXXXXXXXXXXXXXXXXXXXXXXXXXXXXXXXXXXXXXXXXXXXXXXXXXXXXXXXXXXXXXXXXXXXXXXXXXXXXXXXXXXXXXXWVRQAPGKGLEWVGXXXXXXXXXXXXXXXXXXXXXXXXXXXXXXXXXXXXXXXXXXXXXXXXXXXXXXXXXXXXXXXXXXXXXXXXXXXXXXXXXXXXXXXXXXXXXXXXXXXXRFTISRDTSKNTVYLQMNSLRAEDTAVYYCARXXXXXXXXXXXXXXXXXXXXXXXXXXXXXXXXXXXXXXXXXXXXXXXXXXXXXXXXXXXXXXXXXXXXXXXXXXXXXXXXXXXXXXXXXXXXXXXXXXXXWGQGTLVTVSS

SEQ ID NO: 174 - protein, 783 aa, Artificial Sequence
  recombinant scFv - acceptor sequence
  CDR (24)..(123): Al least 3 and up to 50 amino acids can be present.
  CDR (139)..(238): Al least 3 and up to 50 amino acids can be present.
  CDR (271)..(370): Al least 3 and up to 50 amino acids can be present.
  CDR (427)..(526): Al least 3 and up to 50 amino acids can be present.
  CDR (541)..(640): Al least 3 and up to 50 amino acids can be present.
  CDR (673)..(772): Al least 3 and up to 50 amino acids can be present.
EIVMTQSPSTLSASVGDRVIITCXXXXXXXXXXXXXXXXXXXXXXXXXXXXXXXXXXXXXXXXXXXXXXXXXXXXXXXXXXXXXXXXXXXXXXXXXXXXXXXXXXXXXXXXXXXXXXXXXXXXWYQQKPGKAPKLLIYXXXXXXXXXXXXXXXXXXXXXXXXXXXXXXXXXXXXXXXXXXXXXXXXXXXXXXXXXXXXXXXXXXXXXXXXXXXXXXXXXXXXXXXXXXXXXXXXXXXXGVPSRFSGSGSGTEFTLTISSLQPDDFATYYCXXXXXXXXXXXXXXXXXXXXXXXXXXXXXXXXXXXXXXXXXXXXXXXXXXXXXXXXXXXXXXXXXXXXXXXXXXXXXXXXXXXXXXXXXXXXXXXXXXXXFGQGTKLTVLGGGGGSGGGGSGGGGSGGGGSEVQLVESGGGLVQPGGSLRLSCTVSXXXXXXXXXXXXXXXXXXXXXXXXXXXXXXXXXXXXXXXXXXXXXXXXXXXXXXXXXXXXXXXXXXXXXXXXXXXXXXXXXXXXXXXXXXXXXXXXXXXXWVRQAPGKGLEWVGXXXXXXXXXXXXXXXXXXXXXXXXXXXXXXXXXXXXXXXXXXXXXXXXXXXXXXXXXXXXXXXXXXXXXXXXXXXXXXXXXXXXXXXXXXXXXXXXXXXXRFTISKDTSKNTVYLQMNSLRAEDTAVYYCARXXXXXXXXXXXXXXXXXXXXXXXXXXXXXXXXXXXXXXXXXXXXXXXXXXXXXXXXXXXXXXXXXXXXXXXXXXXXXXXXXXXXXXXXXXXXXXXXXXXXWGQGTLVTVSS

SEQ ID NO: 175 - protein, 248 aa, Artificial Sequence
  recombinant scFv
EIVMTQSPSTLSASVGDRVIITCQASQSIGSSLAWYQQKPGKAPKLLIYTAANLASGVPSRFSGSRSGAEFTLTISSLQPDDFATYYCQNFATSDTVTFGQGTKLTVLGGGGGSGGGGSGGGGSGGGGSEVQLVESGGGLVQPGGSLRLSCKASGFSLNTNYWMCWVRQAPGKGLEWVGCMYTGSYNRAYYASWAKGRFTSSKDTSKNTVYLQMNSLRAEDTAVYYCAKGSNWYSDLWGQGTLVTVSS

SEQ ID NO: 176 - protein, 251 aa, Artificial Sequence
  recombinant scFv
EIVMTQSPSTLSASVGDRVIITCQASQSINIWLSWYQQKPGKAPKLLIYRASTLASGVPSRFSGSGSGTEFTLTISSLQPDDFATYYCQANYAYSAGYGAAFGQGTKLTVLGGGGGSGGGGSGGGGSGGGGSEVQLVESGGGLVQPGGSLRLSCTVSGFSLNTYYMNWVRQAPGKGLEWVGIIAPDDTTYYASWAKSRSTISRDTSKNTVYLQMNSLRAEDTAVYYCARSGDTTAWGADIWGQGTLVTVSS

SEQ ID NO: 177 - protein, 250 aa, Artificial Sequence
  recombinant scFv
EIVMTQSPSTLSASVGDRVIITCQADQSIYIWLSWYQQKPGKAPKLLIYKASTLESGVPSRFSGSGSGAEFTLTISSLQPDDFATYYCQNNAHYSTNGGTFGQGTKLTVLGGGGGSGGGGSGGGGSGGGGSEVQLVESGGGLVQPGGSLRLSCAASGFSLSDYYMCWVRQAPGKGLEWVSCLDYFGSTDDASWAKGRFTISRDNSKNTLYLQMNSLRAEDTAVYYCAKTDDSRGWGLNIWGQGTLVTVSS

SEQ ID NO: 178 - protein, 251 aa, Artificial Sequence
  recombinant scFv
EIVMTQSPSTLSASVGDRVIITCQASEIIHSWLAWYQQKPGKAPKLLIYLASTLASGVPSRFSGSGSGAEFTLTISSLQPDDFATYYCQNVYLASTNGANFGQGTKLTVLGGGGGSGGGGSGGGGSGGGGSEVQLVESGGGLVQPGGSLRLSCAASGFSLTDYYYMTWVRQAPGKGLEWVSFIDPDDDPYYATWAKGRFTISRDNSKNTLYLQMNSLRAEDTAVYYCAKGDHNSGWGLDIWGQGTLVTVSS

SEQ ID NO: 179 - protein, 251 aa, Artificial Sequence
  recombinant scFv
EIVMTQSPSTLSASVGDRVIITCQASEIIHSWLAWYQQKPGKAPKLLIYLASTLASGVPSRFSGSGSGTQFTLTISSLQPDDFATYYCQNVYLASTNGANFGQGTKLTVLGGGGGSGGGGSGGGGSGGGGSEVQLVESGGGLVQPGGSLRLSCTASGFSLTDYYYMTWVRQAPGKGLEWVGFIDPDDDPYYATWAKGRFTISRDTSKNTVYLQMNSLRAEDTAVYYCAGGDHNSGWGLDIWGQGTLVTVSS

SEQ ID NO: 180 - protein, 251 aa, Artificial Sequence
  recombinant scFv
EIVMTQSPSTLSASVGDRVIITCQASEIIHSWLAWYQQKPGKAPKLLIYLASTLASGVPSRFSGSGSGAEFTLTISSLQPDDFATYYCQNVYLASTNGANFGQGTKLTVLGGGGGSGGGGSGGGGSGGGGSEVQLVESGGGLVQPGGSLRLSCTASGFSLTDYYYMTWVRQAPGKGLEWVGFIDPDDDPYYATWAKGRFTISRDTSKNTVYLQMNSLRAEDTAVYYCAGGDHNSGWGLDIWGQGTLVTVSS